European Patent Application EP 4 644 394 A2, published November 5, 2025. Title: ANTIVIRAL COMPOUNDS. Applicant: GILEAD SCIENCES, INC. Application EP Herewith. The sequence listing filed with the application follows.

SEQUENCE LISTING (1 sequence)

SEQ ID NO: 1 - RNA, 244 nt, synthetic construct
  misc_feature 1..244: note = Description of Artificial Sequence: Synthetic polynucleotide
  source 1..244: mol_type = other RNA
tcagtcagtcagtcagtcagtcagtcagtcagtcagtcagtcagtcagtcagtcagtcagtcagtcagtcagtcagtcagtccaagtccaagtccaagtccaagtccaagtccaagtccaagtccaagtccaagtccaagtccaagtccaagtccaagtccaagtcagtcagtcagtcagtcagtcagtcagtcagtcagtcagtcagtcagtcagtcagtcagtcagtcagtcagtcagtcag